European Patent Application EP 4 541 822 A2, published April 23, 2025. Title: Phase Change Adjusting Kit and Use Thereof. Applicant: Tsinghua University. Application IB PCT/CN2023/000076, filed June 16, 2023. The sequence listing filed with the application follows.

SEQUENCE LISTING (54 sequences)

SEQ ID NO: 1 - DNA, 738 bp, synthetic construct
  source 1..738: mol_type = other DNA
atgaaacatcatcatcatcatcatcatgaaaacctgtattttcagggcgccatgagcagcaaagtcgatgtaattgacttaacgatcgaatctagcagcgatgaagaagaagatccaccggctaaacgtgggggctcagggggttctggcggttcaggcggcagtaaagttgacgtgattgacctcaccatcgaaagcagtagcgacgaggaagaagatccaccagcaaaacgcggagggagcgggggcagcggcggcagcggcggatctaaagtggacgttatcgatctgacgatcgaaagcagtagcgatgaggaagaggacccgccggcgaaacggggcgccatgaaaggcggtagcggtggcagcggtggtagcggcggctccatgagcagcaaagtcgatgtaattgacttaacgatcgaatctagcagcgatgaagaagaagatccaccggctaaacgtgggggctcagtgggttctggcggttcaggcggcagtaaagttgacgtgattgacctcaccatcgaaagcagtagcgacgaggaagaagatccaccagcaaaacgcggagggagcgggggcagcggcggcaggggcggatctaaagtggacgttatcgatctgacgatcgaaagcagtagcgatgaggaagaggacccgccggcgaaacggggcgccatgaggtgctggggcggtagcggtggcagcggtggtagcggcggctccatggggtaa

SEQ ID NO: 2 - protein, 245 aa, synthetic construct
MKHHHHHHHENLYFQGAMSSKVDVIDLTIESSSDEEEDPPAKRGGSGGSGGSGGSKVDVIDLTIESSSDEEEDPPAKRGGSGGSGGSGGSKVDVIDLTIESSSDEEEDPPAKRGAMKGGSGGSGGSGGSMSSKVDVIDLTIESSSDEEEDPPAKRGGSVGSGGSGGSKVDVIDLTIESSSDEEEDPPAKRGGSGGSGGRGGSKVDVIDLTIESSSDEEEDPPAKRGAMRCWGGSGGSGGSGGSMG

SEQ ID NO: 3 - DNA, 1656 bp, synthetic construct
  source 1..1656: mol_type = other DNA
atgaaacatcatcatcatcatcatcatgaaaacctgtattttcagggcgaaaacctgtattttcagggcgccatgagaatgtcagaagagaagcctaaggagggcgtgaaaaccgagaatgaccacattaacttgaaggttgctggacaggatgggtccgtggttcagttcaaaattaaacgccacacaccgttgtcgaaactgatgaaagcgtactgcgaacgccagggtctttctatgcgtcagattcgcttccgctttgatggtcaaccgattaatgaaacggacacgccggcacagctggagatggaggatgaagacactatcgacgtatttcagcagcagaccgtcgtagggggctccggcggaagcggggggtcgggaggttccatgagcgaagagaaaccaaaagaaggagttaaaaccgaaaacgaccatatcaacctgaaggtcgccggtcaggacggctcagtcgtgcagttcaagattaaacgtcataccccattaagtaagctgatgaaggcgtattgtgagcgccaaggcttgtcgatgcgccagattcgttttcgctttgatggtcagccaatcaacgaaaccgacaccccggcgcagctggaaatggaagatgaagataccatcgatgtgttccaacagcaaacggttgttggcggaagcggcgggagcggtggtagcgggggttctatgtccgaagaaaaaccgaaagagggtgtgaagactgaaaacgaccacattaatctgaaggtggcgggccaggacggttccgttgttcagtttaaaatcaaacgtcacaccccgctgtcgaaactgatgaaagcctattgcgaacgtcaagggctgagcatgcgtcaaattcgttttcgctttgatggtcagccaatcaacgaaaccgatacaccggcgcagctggagatggaagacgaggacaccattgacgtcttccagcaacaaactgtagtgggtggctccggtggctctggtgggtctggtggctcgatgagtgaggaaaaacccaaagaaggcgtcaagactgagaacgatcatattaacctgaaagtcgcgggtcaagatggttcagtggtgcagttcaaaattaaacgccacaccccgctgtcaaagctgatgaaagcctattgtgagcgtcaaggtctgtcgatgcgccagatccgctttcgctttgatggtcagccaatcaacgagacagacactccggcacaactggagatggaagatgaagacaccatcgatgtttttcaacagcagaccgtggtgggagggagcggcggtagcgggggatcaggtggtagtatgtctgaggaaaagccgaaggaaggggtaaagaccgaaaatgatcacattaatctgaaagttgcgggccaagatggtagtgtagtgcaatttaaaatcaagcgtcacaccccgttatctaaactgatgaaagcatattgcgaacgccaaggcctgtctatgcgccagattcgctttcgctttgacgggcaaccaattaatgaaacggacaccccggcacaactggaaatggaagacgaggatactattgacgtgtttcagcaacagacagtggtcgccatgaaaggcggtagcggtggcagcggtggtagcggcggctccatgggctaa

SEQ ID NO: 4 - protein, 551 aa, synthetic construct
MKHHHHHHHENLYFQGENLYFQGAMRMSEEKPKEGVKTENDHINLKVAGQDGSVVQFKIKRHTPLSKLMKAYCERQGLSMRQIRFRFDGQPINETDTPAQLEMEDEDTIDVFQQQTVVGGSGGSGGSGGSMSEEKPKEGVKTENDHINLKVAGQDGSVVQFKIKRHTPLSKLMKAYCERQGLSMRQIRFRFDGQPINETDTPAQLEMEDEDTIDVFQQQTVVGGSGGSGGSGGSMSEEKPKEGVKTENDHINLKVAGQDGSVVQFKIKRHTPLSKLMKAYCERQGLSMRQIRFRFDGQPINETDTPAQLEMEDEDTIDVFQQQTVVGGSGGSGGSGGSMSEEKPKEGVKTENDHINLKVAGQDGSVVQFKIKRHTPLSKLMKAYCERQGLSMRQIRFRFDGQPINETDTPAQLEMEDEDTIDVFQQQTVVGGSGGSGGSGGSMSEEKPKEGVKTENDHINLKVAGQDGSVVQFKIKRHTPLSKLMKAYCERQGLSMRQIRFRFDGQPINETDTPAQLEMEDEDTIDVFQQQTVVAMKGGSGGSGGSGGSMG

SEQ ID NO: 5 - DNA, 825 bp, synthetic construct
  source 1..825: mol_type = other DNA
atgaaacatcatcatcatcatcatcatgaaaacctgtattttcagggcgccatgagcagcaaagtcgatgtaattgacttaacgatcgaatctagcagcgatgaagaagaagatccaccggctaaacgtgggggctcagggggttctggcggttcaggcggcagtaaagttgacgtgattgacctcaccatcgaaagcagtagcgacgaggaagaagatccaccagcaaaacgcggagggagcgggggcagcggcggcagcggcggatctaaagtggacgttatcgatctgacgatcgaaagcagtagcgatgaggaagaggacccgccggcgaaacggggcgccatgaaaggcggtagcggtggcagcggtggtagcggcggctccatgagcagcaaagtcgatgtaattgacttaacgatcgaatctagcagcgatgaagaagaagatccaccggctaaacgtgggggctcagtgggttctggcggttcaggcggcagtaaagttgacgtgattgacctcaccatcgaaagcagtagcgacgaggaagaagatccaccagcaaaacgcggagggagcgggggcagcggcggcaggggcggatctaaagtggacgttatcgatctgacgatcgaaagcagtagcgatgaggaagaggacccgccggcgaaacggggcgccatgaggtgctggggcggtagcggtggcagcggtggtagcggcggctccatggggatgtgctaccgtaaatgccgtggtggtcgtcgttggtgctaccagaaatgcggtggttctggtggttctggtggttctggtggttcttaa

SEQ ID NO: 6 - protein, 274 aa, synthetic construct
MKHHHHHHHENLYFQGAMSSKVDVIDLTIESSSDEEEDPPAKRGGSGGSGGSGGSKVDVIDLTIESSSDEEEDPPAKRGGSGGSGGSGGSKVDVIDLTIESSSDEEEDPPAKRGAMKGGSGGSGGSGGSMSSKVDVIDLTIESSSDEEEDPPAKRGGSVGSGGSGGSKVDVIDLTIESSSDEEEDPPAKRGGSGGSGGRGGSKVDVIDLTIESSSDEEEDPPAKRGAMRCWGGSGGSGGSGGSMGMCYRKCRGGRRWCYQKCGGSGGSGGSGGS

SEQ ID NO: 7 - DNA, 2160 bp, synthetic construct
  source 1..2160: mol_type = other DNA
atgaaacatcatcatcatcatcatcatgaaaacctgtattttcagggcgaaaacctgtattttcagggcgccatgagaatgtcagaagagaagcctaaggagggcgtgaaaaccgagaatgaccacattaacttgaaggttgctggacaggatgggtccgtggttcagttcaaaattaaacgccacacaccgttgtcgaaactgatgaaagcgtactgcgaacgccagggtctttctatgcgtcagattcgcttccgctttgatggtcaaccgattaatgaaacggacacgccggcacagctggagatggaggatgaagacactatcgacgtatttcagcagcagaccgtcgtagggggctccggcggaagcggggggtcgggaggttccatgagcgaagagaaaccaaaagaaggagttaaaaccgaaaacgaccatatcaacctgaaggtcgccggtcaggacggctcagtcgtgcagttcaagattaaacgtcataccccattaagtaagctgatgaaggcgtattgtgagcgccaaggcttgtcgatgcgccagattcgttttcgctttgatggtcagccaatcaacgaaaccgacaccccggcgcagctggaaatggaagatgaagataccatcgatgtgttccaacagcaaacggttgttggcggaagcggcgggagcggtggtagcgggggttctatgtccgaagaaaaaccgaaagagggtgtgaagactgaaaacgaccacattaatctgaaggtggcgggccaggacggttccgttgttcagtttaaaatcaaacgtcacaccccgctgtcgaaactgatgaaagcctattgcgaacgtcaagggctgagcatgcgtcaaattcgttttcgctttgatggtcagccaatcaacgaaaccgatacaccggcgcagctggagatggaagacgaggacaccattgacgtcttccagcaacaaactgtagtgggtggctccggtggctctggtgggtctggtggctcgatgagtgaggaaaaacccaaagaaggcgtcaagactgagaacgatcatattaacctgaaagtcgcgggtcaagatggttcagtggtgcagttcaaaattaaacgccacaccccgctgtcaaagctgatgaaagcctattgtgagcgtcaaggtctgtcgatgcgccagatccgctttcgctttgatggtcagccaatcaacgagacagacactccggcacaactggagatggaagatgaagacaccatcgatgtttttcaacagcagaccgtggtgggagggagcggcggtagcgggggatcaggtggtagtatgtctgaggaaaagccgaaggaaggggtaaagaccgaaaatgatcacattaatctgaaagttgcgggccaagatggtagtgtagtgcaatttaaaatcaagcgtcacaccccgttatctaaactgatgaaagcatattgcgaacgccaaggcctgtctatgcgccagattcgctttcgctttgacgggcaaccaattaatgaaacggacaccccggcacaactggaaatggaagacgaggatactattgacgtgtttcagcaacagacagtggtcgccatgaaaggcggtagcggtggcagcggtggtagcggcggctccatgggcgttcgtgaacgtggtccgcagcgtgttgctgctcacatcaccggtacccgtggtcgttctaacaccctgtcttctccgaactctaaaaacgaaaaagctctgggtcgtaaaatcaactcttgggaatcttctcgttctggtcactctttcctgtctaacctgcacctgcgtaacggtgaactggttatccacgaaaaaggtttctactacatctactctcagacctacttccgtttccaggaagaaatcaaagaaaacaccaaaaacgacaaacagatggttcagtacatctacaaatacacctcttacccggacccgatcctgctgatgaaatctgctcgtaactcttgctggtctaaagacgctgaatacggtctgtactctatctaccagggtggtatcttcgaactgaaagaaaacgaccgtatcttcgtttctgttaccaacgaacacctgatcgacatggaccacgaagcttctttttttggtgcgttcctggttggctaa

SEQ ID NO: 8 - protein, 719 aa, synthetic construct
MKHHHHHHHENLYFQGENLYFQGAMRMSEEKPKEGVKTENDHINLKVAGQDGSVVQFKIKRHTPLSKLMKAYCERQGLSMRQIRFRFDGQPINETDTPAQLEMEDEDTIDVFQQQTVVGGSGGSGGSGGSMSEEKPKEGVKTENDHINLKVAGQDGSVVQFKIKRHTPLSKLMKAYCERQGLSMRQIRFRFDGQPINETDTPAQLEMEDEDTIDVFQQQTVVGGSGGSGGSGGSMSEEKPKEGVKTENDHINLKVAGQDGSVVQFKIKRHTPLSKLMKAYCERQGLSMRQIRFRFDGQPINETDTPAQLEMEDEDTIDVFQQQTVVGGSGGSGGSGGSMSEEKPKEGVKTENDHINLKVAGQDGSVVQFKIKRHTPLSKLMKAYCERQGLSMRQIRFRFDGQPINETDTPAQLEMEDEDTIDVFQQQTVVGGSGGSGGSGGSMSEEKPKEGVKTENDHINLKVAGQDGSVVQFKIKRHTPLSKLMKAYCERQGLSMRQIRFRFDGQPINETDTPAQLEMEDEDTIDVFQQQTVVAMKGGSGGSGGSGGSMGVRERGPQRVAAHITGTRGRSNTLSSPNSKNEKALGRKINSWESSRSGHSFLSNLHLRNGELVIHEKGFYYIYSQTYFRFQEEIKENTKNDKQMVQYIYKYTSYPDPILLMKSARNSCWSKDAEYGLYSIYQGGIFELKENDRIFVSVTNEHLIDMDHEASFFGAFLVG

SEQ ID NO: 9 - DNA, 1122 bp, synthetic construct
  source 1..1122: mol_type = other DNA
atgaaacatcatcatcatcatcatcatgaaaacctgtattttcagggcgccatgagcagcaaagtcgatgtaattgacttaacgatcgaatctagcagcgatgaagaagaagatccaccggctaaacgtgggggctcagggggttctggcggttcaggcggcagtaaagttgacgtgattgacctcaccatcgaaagcagtagcgacgaggaagaagatccaccagcaaaacgcggagggagcgggggcagcggcggcagcggcggatctaaagtggacgttatcgatctgacgatcgaaagcagtagcgatgaggaagaggacccgccggcgaaacggggcgccatgaaaggcggtagcggtggcagcggtggtagcggcggctccatgagcagcaaagtcgatgtaattgacttaacgatcgaatctagcagcgatgaagaagaagatccaccggctaaacgtgggggctcagtgggttctggcggttcaggcggcagtaaagttgacgtgattgacctcaccatcgaaagcagtagcgacgaggaagaagatccaccagcaaaacgcggagggagcgggggcagcggcggcaggggcggatctaaagtggacgttatcgatctgacgatcgaaagcagtagcgatgaggaagaggacccgccggcgaaacggggcgccatgaggtgctggggcggtagcggtggcagcggtggtagcggcggctccatgggggaagttcagctgatggaatctggtggtggtctggttcaggctggtggttctctgcgtctgtcttgcgctgcttctggtcgtaccttcaacaactacgctatgggttggttccgtcgtgctccgaaaggtgaacgtgaattcgttgctgctatcacccgttctggtgttcgttctggtgtttctgctatctacggtgactctgttaaagaccgtttcaccatctctcgtgacaacgctaaaaacaccctgtacctgcagatgaactctctgaaaccggaagacaccgctgtttacacctgcgctgcttctgctatcggttctggtgcgctccgtaggttcgaatacgactactctggtcagggtactcaggttaccgtaagctcttaa

SEQ ID NO: 10 - protein, 373 aa, synthetic construct
MKHHHHHHHENLYFQGAMSSKVDVIDLTIESSSDEEEDPPAKRGGSGGSGGSGGSKVDVIDLTIESSSDEEEDPPAKRGGSGGSGGSGGSKVDVIDLTIESSSDEEEDPPAKRGAMKGGSGGSGGSGGSMSSKVDVIDLTIESSSDEEEDPPAKRGGSVGSGGSGGSKVDVIDLTIESSSDEEEDPPAKRGGSGGSGGRGGSKVDVIDLTIESSSDEEEDPPAKRGAMRCWGGSGGSGGSGGSMGEVQLMESGGGLVQAGGSLRLSCAASGRTFNNYAMGWFRRAPKGEREFVAAITRSGVRSGVSAIYGDSVKDRFTISRDNAKNTLYLQMNSLKPEDTAVYTCAASAIGSGALRRFEYDYSGQGTQVTVSS

SEQ ID NO: 11 - DNA, 2022 bp, synthetic construct
  source 1..2022: mol_type = other DNA
atgaaacatcatcatcatcatcatcatgaaaacctgtattttcagggcgaaaacctgtattttcagggcgccatgagaatgtcagaagagaagcctaaggagggcgtgaaaaccgagaatgaccacattaacttgaaggttgctggacaggatgggtccgtggttcagttcaaaattaaacgccacacaccgttgtcgaaactgatgaaagcgtactgcgaacgccagggtctttctatgcgtcagattcgcttccgctttgatggtcaaccgattaatgaaacggacacgccggcacagctggagatggaggatgaagacactatcgacgtatttcagcagcagaccgtcgtagggggctccggcggaagcggggggtcgggaggttccatgagcgaagagaaaccaaaagaaggagttaaaaccgaaaacgaccatatcaacctgaaggtcgccggtcaggacggctcagtcgtgcagttcaagattaaacgtcataccccattaagtaagctgatgaaggcgtattgtgagcgccaaggcttgtcgatgcgccagattcgttttcgctttgatggtcagccaatcaacgaaaccgacaccccggcgcagctggaaatggaagatgaagataccatcgatgtgttccaacagcaaacggttgttggcggaagcggcgggagcggtggtagcgggggttctatgtccgaagaaaaaccgaaagagggtgtgaagactgaaaacgaccacattaatctgaaggtggcgggccaggacggttccgttgttcagtttaaaatcaaacgtcacaccccgctgtcgaaactgatgaaagcctattgcgaacgtcaagggctgagcatgcgtcaaattcgttttcgctttgatggtcagccaatcaacgaaaccgatacaccggcgcagctggagatggaagacgaggacaccattgacgtcttccagcaacaaactgtagtgggtggctccggtggctctggtgggtctggtggctcgatgagtgaggaaaaacccaaagaaggcgtcaagactgagaacgatcatattaacctgaaagtcgcgggtcaagatggttcagtggtgcagttcaaaattaaacgccacaccccgctgtcaaagctgatgaaagcctattgtgagcgtcaaggtctgtcgatgcgccagatccgctttcgctttgatggtcagccaatcaacgagacagacactccggcacaactggagatggaagatgaagacaccatcgatgtttttcaacagcagaccgtggtgggagggagcggcggtagcgggggatcaggtggtagtatgtctgaggaaaagccgaaggaaggggtaaagaccgaaaatgatcacattaatctgaaagttgcgggccaagatggtagtgtagtgcaatttaaaatcaagcgtcacaccccgttatctaaactgatgaaagcatattgcgaacgccaaggcctgtctatgcgccagattcgctttcgctttgacgggcaaccaattaatgaaacggacaccccggcacaactggaaatggaagacgaggatactattgacgtgtttcagcaacagacagtggtcgccatgaaaggcggtagcggtggcagcggtggtagcggcggctccatgggcgaagttcagctgctggaatctggtggtggtctggttcagccgggtggttctctgcgtctgtcttgcgctgcttctggtaccttcgacaaaatcaacaacatgggttggtaccgtcaggctccgggtaaacagcgtgacctggttgctcagatcaccccgggtggtatcaccgactacgctgactctgttaaaggtcgtttcaccatctctcgtgacaactctaaaaacaccctgtacctgcagatgaactctctgcgtccggaagacaccgctgtttactactgcaacgctgaaatcctgaaacgtgcttacatcgacgtttacgttaactactggggtcagggtactctcgttaccgtaagctcttaa

SEQ ID NO: 12 - protein, 673 aa, synthetic construct
MKHHHHHHHENLYFQGENLYFQGAMRMSEEKPKEGVKTENDHINLKVAGQDGSVVQFKIKRHTPLSKLMKAYCERQGLSMRQIRFRFDGQPINETDTPAQLEMEDEDTIDVFQQQTVVGGSGGSGGSGGSMSEEKPKEGVKTENDHINLKVAGQDGSVVQFKIKRHTPLSKLMKAYCERQGLSMRQIRFRFDGQPINETDTPAQLEMEDEDTIDVFQQQTVVGGSGGSGGSGGSMSEEKPKEGVKTENDHINLKVAGQDGSVVQFKIKRHTPLSKLMKAYCERQGLSMRQIRFRFDGQPINETDTPAQLEMEDEDTIDVFQQQTVVGGSGGSGGSGGSMSEEKPKEGVKTENDHINLKVAGQDGSVVQFKIKRHTPLSKLMKAYCERQGLSMRQIRFRFDGQPINETDTPAQLEMEDEDTIDVFQQQTVVGGSGGSGGSGGSMSEEKPKEGVKTENDHINLKVAGQDGSVVQFKIKRHTPLSKLMKAYCERQGLSMRQIRFRFDGQPINETDTPAQLEMEDEDTIDVFQQQTVVAMKGGSGGSGGSGGSMGEVQLLESGGGLVQPGGSLRLSCAASGTFDKINNMGWYRQAPGKQRDLVAQITPGGITDYADSVKGRFTISRDNSKNTLYLQMNSLRPEDTAVYYCNAEILKRAYIDVYVNYWGQGTLVTVSS

SEQ ID NO: 13 - DNA, 447 bp, synthetic construct
  source 1..447: mol_type = other DNA
atgaaacatcatcatcatcatcatcatgaaaacctgtattttcagggcgccatgagcagcgaagttcagctgatggaatctggtggtggtctggttcaggctggtggttctctgcgtctgtcttgcgctgcttctggtcgtaccttcaacaactacgctatgggttggttccgtcgtgctccgaaaggtgaacgtgaattcgttgctgctatcacccgttctggtgttcgttctggtgtttctgctatctacggtgactctgttaaagaccgtttcaccatctctcgtgacaacgctaaaaacaccctgtacctgcagatgaactctctgaaaccggaagacaccgctgtttacacctgcgctgcttctgctatcggttctggtgcgctccgtaggttcgaatacgactactctggtcagggtactcaggttaccgtaagctcttaa

SEQ ID NO: 14 - protein, 148 aa, synthetic construct
MKHHHHHHHENLYFQGAMSSEVQLMESGGGLVQAGGSLRLSCAASGRTFNNYAMGWFRRAPKGEREFVAAITRSGVRSGVSAIYGDSVKDRFTISRDNAKNTLYLQMNSLKPEDTAVYTCAASAIGSGALRRFEYDYSGQGTQVTVSS

SEQ ID NO: 15 - DNA, 447 bp, synthetic construct
  source 1..447: mol_type = other DNA
atgaaacatcatcatcatcatcatcatgaaaacctgtattttcagggcgaaaacctgtattttcagggcgccatgagagaagttcagctgctggaatctggtggtggtctggttcagccgggtggttctctgcgtctgtcttgcgctgcttctggtaccttcgacaaaatcaacaacatgggttggtaccgtcaggctccgggtaaacagcgtgacctggttgctcagatcaccccgggtggtatcaccgactacgctgactctgttaaaggtcgtttcaccatctctcgtgacaactctaaaaacaccctgtacctgcagatgaactctctgcgtccggaagacaccgctgtttactactgcaacgctgaaatcctgaaacgtgcttacatcgacgtttacgttaactactggggtcagggtactctcgttaccgtaagctcttaa

SEQ ID NO: 16 - protein, 148 aa, synthetic construct
MKHHHHHHHENLYFQGENLYFQGAMREVQLLESGGGLVQPGGSLRLSCAASGTFDKINNMGWYRQAPGKQRDLVAQITPGGITDYADSVKGRFTISRDNSKNTLYLQMNSLRPEDTAVYYCNAEILKRAYIDVYVNYWGQGTLVTVSS

SEQ ID NO: 17 - DNA, 774 bp, synthetic construct
  source 1..774: mol_type = other DNA
atgaaacatcatcatcatcatcatcatgaaaacctgtattttcagggcgccatgaaagtggacgttatcgatctgacgatcgaaagcagtagcgatgaggaagaggacccgccggcgaaacggggagggagcgggggcagcggcggcagcggcggatccatgatgaaagtggacgttatcgatctgacgatcgaaagcagtagcgatgaggaagaggacccgccggcgaaacggggagggagcgggggcagcggcggcagcggcggatccatgatgaaagtggacgttatcgatctgacgatcgaaagcagtagcgatgaggaagaggacccgccggcgaaacggggagggagcgggggcagcggcggcagcggcggatccatgggggaagttcagctgatggaatctggtggtggtctggttcaggctggtggttctctgcgtctgtcttgcgctgcttctggtcgtaccttcaacaactacgctatgggttggttccgtcgtgctccgaaaggtgaacgtgaattcgttgctgctatcacccgttctggtgttcgttctggtgtttctgctatctacggtgactctgttaaagaccgtttcaccatctctcgtgacaacgctaaaaacaccctgtacctgcagatgaactctctgaaaccggaagacaccgctgtttacacctgcgctgcttctgctatcggttctggtgcgctccgtaggttcgaatacgactactctggtcagggtactcaggttaccgtaagctcttaa

SEQ ID NO: 18 - protein, 257 aa, synthetic construct
MKHHHHHHHENLYFQGAMKVDVIDLTIESSSDEEEDPPAKRGGSGGSGGSGGSMMKVDVIDLTIESSSDEEEDPPAKRGGSGGSGGSGGSMMKVDVIDLTIESSSDEEEDPPAKRGGSGGSGGSGGSMGEVQLMESGGGLVQAGGSLRLSCAASGRTFNNYAMGWFRRAPKGEREFVAAITRSGVRSGVSAIYGDSVKDRFTISRDNAKNTLYLQMNSLKPEDTAVYTCAASAIGSGALRRFEYDYSGQGTQVTVSS

SEQ ID NO: 19 - DNA, 1373 bp, synthetic construct
  source 1..1373: mol_type = other DNA
atgaaacatcatcatcatcatcatcatgaaaacctgtattttcagggcgccatgatgtcagaagagaagcctaaggagggcgtgaaaaccgagaatgaccacattaacttgaaggttgctggacaggatgggtccgtggttcagttcaaaattaaacgccacaccccgctgtcaaagctgatgaaagcctattgtgagcgtcaaggtctgtcgatgcgccagatccgctttcgctttgatggtcagccaatcaacgagacagacactccggcacaactggagatggaagatgaagacaccatcgatgtttttcaacagcagaccgtggtgggagggagcggcggtagcgggggatcaggtggtagtccaatgtcagaagagaagcctaaggagggcgtgaaaaccgagaatgaccacattaacttgaaggttgctggacaggatgggtccgtggttcagttcaaaattaaacgccacaccccgctgtcaaagctgatgaaagcctattgtgagcgtcaaggtctgtcgatgcgccagatccgctttcgctttgatggtcagccaatcaacgagacagacactccggcacaactggagatggaagatgaagacaccatcgatgtttttcaacagcagaccgtggtgggagggagcggcggtagcgggggatcaggtggtagtccaatgtcagaagagaagcctaaggagggcgtgaaaaccgagaatgaccacattaacttgaaggttgctggacaggatgggtccgtggttcagttcaaaattaaacgccacaccccgctgtcaaagctgatgaaagcatattgcgaacgccaaggcctgtctatgcgccagattcgctttcgctttgatggtcagccaatcaacgagacagacactccggcacaactggagatggaagatgaagacaccatcgatgtttttcaacagcagaccgtggtgggagggagcggcggtagcgggggatcaggtggtagtgccatggggaagttcagctgctggaatctggtggtggtctggttcagccgggtggttctctgcgtctgtcttgcgctgcttctggtaccttcgacaaaatcaacaacatgggttggtaccgtcaggctccgggtaaacagcgtgacctggttgctcagatcaccccgggtggtatcaccgactacgctgactctgttaaaggtcgtttcaccatctctcgtgacaactctaaaaacaccctgtacctgcagatgaactctctgcgtccggaagacaccgctgtttactactgcaacgctgaaatcctgaaacgtgcttacatcgacgtttacgttaactactggggtcagggtactctcgttaccgtaagctcttaa

SEQ ID NO: 20 - protein, 457 aa, synthetic construct
MKHHHHHHHENLYFQGAMMSEEKPKEGVKTENDHINLKVAGQDGSVVQFKIKRHTPLSKLMKAYCERQGLSMRQIRFRFDGQPINETDTPAQLEMEDEDTIDVFQQQTVVGGSGGSGGSGGSPMSEEKPKEGVKTENDHINLKVAGQDGSVVQFKIKRHTPLSKLMKAYCERQGLSMRQIRFRFDGQPINETDTPAQLEMEDEDTIDVFQQQTVVGGSGGSGGSGGSPMSEEKPKEGVKTENDHINLKVAGQDGSVVQFKIKRHTPLSKLMKAYCERQGLSMRQIRFRFDGQPINETDTPAQLEMEDEDTIDVFQQQTVVGGSGGSGGSGGSAMGEVQLLESGGGLVQPGGSLRLSCAASGTFDKINNMGWYRQAPGKQRDLVAQITPGGITDYADSVKGRFTISRDNSKNTLYLQMNSLRPEDTAVYYCNAEILKRAYIDVYVNYWGQGTLVTVSS

SEQ ID NO: 21 - DNA, 390 bp, synthetic construct
  source 1..390: mol_type = other DNA
atgaaacatcatcatcatcatcatcatgaaaacctgtattttcagggcgccatgaaagtggacgttatcgatctgacgatcgaaagcagtagcgatgaggaagaggacccgccggcgaaacggggagggagcgggggcagcggcggcagcggcggatccatgatgaaagtggacgttatcgatctgacgatcgaaagcagtagcgatgaggaagaggacccgccggcgaaacggggagggagcgggggcagcggcggcagcggcggatccatgatgaaagtggacgttatcgatctgacgatcgaaagcagtagcgatgaggaagaggacccgccggcgaaacggggagggagcgggggcagcggcggcagcggcggatccatggggtaa

SEQ ID NO: 22 - protein, 115 aa, synthetic construct
MKHHHHHHHENLYFQGAMKVDVIDLTIESSSDEEEDPPAKRGGSGGSGGSGGSMMKVDVIDLTIESSSDEEEDPPAKRGGSGGSGGSGGSMMKVDVIDLTIESSSDEEEDPPAKR

SEQ ID NO: 23 - DNA, 1005 bp, synthetic construct
  source 1..1005: mol_type = other DNA
atgaaacatcatcatcatcatcatcatgaaaacctgtattttcagggcgccatgatgtcagaagagaagcctaaggagggcgtgaaaaccgagaatgaccacattaacttgaaggttgctggacaggatgggtccgtggttcagttcaaaattaaacgccacaccccgctgtcaaagctgatgaaagcctattgtgagcgtcaaggtctgtcgatgcgccagatccgctttcgctttgatggtcagccaatcaacgagacagacactccggcacaactggagatggaagatgaagacaccatcgatgtttttcaacagcagaccgtggtgggagggagcggcggtagcgggggatcaggtggtagtccaatgtcagaagagaagcctaaggagggcgtgaaaaccgagaatgaccacattaacttgaaggttgctggacaggatgggtccgtggttcagttcaaaattaaacgccacaccccgctgtcaaagctgatgaaagcctattgtgagcgtcaaggtctgtcgatgcgccagatccgctttcgctttgatggtcagccaatcaacgagacagacactccggcacaactggagatggaagatgaagacaccatcgatgtttttcaacagcagaccgtggtgggagggagcggcggtagcgggggatcaggtggtagtccaatgtcagaagagaagcctaaggagggcgtgaaaaccgagaatgaccacattaacttgaaggttgctggacaggatgggtccgtggttcagttcaaaattaaacgccacaccccgctgtcaaagctgatgaaagcctattgtgagcgtcaaggtctgtcgatgcgccagatccgctttcgctttgatggtcagccaatcaacgagacagacactccggcacaactggagatggaagatgaagacaccatcgatgtttttcaacagcagaccgtggtgggagggagcggcggtagcgggggatcaggtggtagtccatggtaa

SEQ ID NO: 24 - protein, 320 aa, synthetic construct
MKHHHHHHHENLYFQGAMMSEEKPKEGVKTENDHINLKVAGQDGSVVQFKIKRHTPLSKLMKAYCERQGLSMRQIRFRFDGQPINETDTPAQLEMEDEDTIDVFQQQTVVGGSGGSGGSGGSPMSEEKPKEGVKTENDHINLKVAGQDGSVVQFKIKRHTPLSKLMKAYCERQGLSMRQIRFRFDGQPINETDTPAQLEMEDEDTIDVFQQQTVVGGSGGSGGSGGSPMSEEKPKEGVKTENDHINLKVAGQDGSVVQFKIKRHTPLSKLMKAYCERQGLSMRQIRFRFDGQPINETDTPAQLEMEDEDTIDVFQQQTVV

SEQ ID NO: 25 - DNA, 891 bp, synthetic construct
  source 1..891: mol_type = other DNA
atgaaacatcatcatcatcatcatcatgaaaacctgtattttcagggtcatatgaaaggcggcagctggggtggtagcaaaaaaaccccgccgccagtgccaccacgcaccaccagcaaaggtggtagcggtggtagcggtggtagcggtggtagtaaaaaaaccccgccaccggtgccgccacgtaccaccagcaaaggtggtagcggtggcagtggtggtagtggtggtagcaaaaaaaccccgccgccagtgccaccacgtaccaccagtaaaggtggtagcggcggtagcggtggtagcggtggtagcaaaaaaaccccgccaccagtgccgccacgcaccaccagtaaaggtggcagtggtggtagcggcggtagcggtggtagtaaaaaaaccccgccaccggtgccgccacgtaccaccagcaaaggcggtagcggtagcaaaaatctgtattttcagggcggtagcggtggcagcggtggtagcggcggctccatggaagttcagctgatggaatctggtggtggtctggttcaggctggtggttctctgcgtctgtcttgcgctgcttctggtcgtaccttcaacaactacgctatgggttggttccgtcgtgctccgaaaggtgaacgtgaattcgttgctgctatcacccgttctggtgttcgttctggtgtttctgctatctacggtgactctgttaaagaccgtttcaccatctctcgtgacaacgctaaaaacaccctgtacctgcagatgaactctctgaaaccggaagacaccgctgtttacacctgcgctgcttctgctatcggttctggtgcgctccgtaggttcgaatacgactactctggtcagggtactcaggttaccgtaagctcttaa

SEQ ID NO: 26 - protein, 296 aa, synthetic construct
MKHHHHHHHENLYFQGHMKGGSWGGSKKTPPPVPPRTTSKGGSGGSGGSGGSKKTPPPVPPRTTSKGGSGGSGGSGGSKKTPPPVPPRTTSKGGSGGSGGSGGSKKTPPPVPPRTTSKGGSGGSGGSGGSKKTPPPVPPRTTSKGGSGSKNLYFQGGSGGSGGSGGSMEVQLMESGGGLVQAGGSLRLSCAASGRTFNNYAMGWFRRAPKGEREFVAAITRSGVRSGVSAIYGDSVKDRFTISRDNAKNTLYLQMNSLKPEDTAVYTCAASAIGSGALRRFEYDYSGQGTQVTVSS

SEQ ID NO: 27 - DNA, 1653 bp, synthetic construct
  source 1..1653: mol_type = other DNA
atgaaacatcatcatcatcatcatcatgaaaacctgtattttcagggccatatggatctgaatatgccggcgtatgtgaaatttaattacatggcggaacgcgaagatgagctgagcctgattaaaggcaccaaagtgattgtgatggaaaagagcagcgatggctggtggcgcggcagctataatggccaagttggttggtttccgagcaattatgtgaccgaagaaggcgatagcccgctggcgagtggtgcgggtggtagcgaaggtggtggtagcgaaggtggtaccagcggtgcgaccgatttgaatatgccggcgtatgtgaaatttaattacatggcggaacgcgaggatgagctgagcctgattaaaggcaccaaagtgattgtgatggaaaagagcagcgatggctggtggcgcggcagctataatggccaagttggctggtttccgagcaattatgtgaccgaagaaggcgatagcccgctggcgagcggtgcgggtggtagcgaaggtggtggcagcgaaggtggtaccagcggtgcgacccatatggatttaaatatgccggcgtatgtgaaattcaactacatggcggaacgcgaggatgagctgagcctgattaaaggcaccaaagtgattgtgatggaaaagagcagcgatggctggtggcgcggcagctataatggccaagttggctggtttccgagcaattatgtgaccgaagaaggcgatagcccgctggcgagcggtgcgggtggtagtgaaggtggcggtagtgaaggcggtaccagcggtgcgaccgatttgaatatgccggcgtatgtgaaatttaattacatggcggaacgcgaggatgagctgagcctgattaaaggcaccaaagtgattgtgatggaaaagagcagcgatggctggtggcgcggcagctataatggccaagttggttggtttccgagcaattatgtgaccgaagaaggcgatagcccgctggcgagtggtgcgggtggtagcgaaggtggtggtagcgaaggtggtaccagcggtgcgaccgatttaaatatgccggcgtatgtgaaatttaattacatggcggaacgcgaggacgagctgagcctgattaaaggcaccaaagtgattgtgatggaaaagagcagcgatggctggtggcgcggcagctataatggccaagtaggctggtttccgagcaattatgtgaccgaagaaggcgatagcccgctgggcggtagcggtggcagcggtggtagcggcggctccatggaagttcagctgctggaatctggtggtggtctggttcagccgggtggttctctgcgtctgtcttgcgctgcttctggtaccttcgacaaaatcaacaacatgggttggtaccgtcaggctccgggtaaacagcgtgacctggttgctcagatcaccccgggtggtatcaccgactacgctgactctgttaaaggtcgtttcaccatctctcgtgacaactctaaaaacaccctgtacctgcagatgaactctctgcgtccggaagacaccgctgtttactactgcaacgctgaaatcctgaaacgtgcttacatcgacgtttacgttaactactggggtcagggtactctcgttaccgtaagctcttaa

SEQ ID NO: 28 - protein, 550 aa, synthetic construct
MKHHHHHHHENLYFQGHMDLNMPAYVKFNYMAEREDELSLIKGTKVIVMEKSSDGWWRGSYNGQVGWFPSNYVTEEGDSPLASGAGGSEGGGSEGGTSGATDLNMPAYVKFNYMAEREDELSLIKGTKVIVMEKSSDGWWRGSYNGQVGWFPSNYVTEEGDSPLASGAGGSEGGGSEGGTSGATHMDLNMPAYVKFNYMAEREDELSLIKGTKVIVMEKSSDGWWRGSYNGQVGWFPSNYVTEEGDSPLASGAGGSEGGGSEGGTSGATDLNMPAYVKFNYMAEREDELSLIKGTKVIVMEKSSDGWWRGSYNGQVGWFPSNYVTEEGDSPLASGAGGSEGGGSEGGTSGATDLNMPAYVKFNYMAEREDELSLIKGTKVIVMEKSSDGWWRGSYNGQVGWFPSNYVTEEGDSPLGGSGGSGGSGGSMEVQLLESGGGLVQPGGSLRLSCAASGTFDKINNMGWYRQAPGKQRDLVAQITPGGITDYADSVKGRFTISRDNSKNTLYLQMNSLRPEDTAVYYCNAEILKRAYIDVYVNYWGQGTLVTVSS

SEQ ID NO: 29 - DNA, 41 bp, synthetic construct
  source 1..41: mol_type = other DNA
actttaataaggagatataccatgaaacatcatcatcatca

SEQ ID NO: 30 - DNA, 40 bp, synthetic construct
  source 1..40: mol_type = other DNA
ttctttaccagactcgagttaccccatggagccgccgcta

SEQ ID NO: 31 - DNA, 43 bp, synthetic construct
  source 1..43: mol_type = other DNA
actttaataaggagatataccatgaaacatcatcatcatcatc

SEQ ID NO: 32 - DNA, 40 bp, synthetic construct
  source 1..40: mol_type = other DNA
ttctttaccagactcgagttagcccatggagccgccgcta

SEQ ID NO: 33 - DNA, 42 bp, synthetic construct
  source 1..42: mol_type = other DNA
actttaataaggagatataccatgaaacatcatcatcatcat

SEQ ID NO: 34 - DNA, 39 bp, synthetic construct
  source 1..39: mol_type = other DNA
ttctttaccagactcgagttaagaaccaccagaaccacc

SEQ ID NO: 35 - DNA, 43 bp, synthetic construct; identical to SEQ ID NO: 31
  source 1..43: mol_type = other DNA

SEQ ID NO: 36 - DNA, 39 bp, synthetic construct
  source 1..39: mol_type = other DNA
ttctttaccagactcgagttagccaaccaggaacgcacc

SEQ ID NO: 37 - DNA, 43 bp, synthetic construct; identical to SEQ ID NO: 31
  source 1..43: mol_type = other DNA

SEQ ID NO: 38 - DNA, 40 bp, synthetic construct
  source 1..40: mol_type = other DNA
ttctttaccagactcgagttaagagcttacggtaacctga

SEQ ID NO: 39 - DNA, 42 bp, synthetic construct; identical to SEQ ID NO: 33
  source 1..42: mol_type = other DNA

SEQ ID NO: 40 - DNA, 39 bp, synthetic construct
  source 1..39: mol_type = other DNA
ttctttaccagactcgagttaagagcttacggtaacgag

SEQ ID NO: 41 - DNA, 42 bp, synthetic construct; identical to SEQ ID NO: 33
  source 1..42: mol_type = other DNA

SEQ ID NO: 42 - DNA, 39 bp, synthetic construct
  source 1..39: mol_type = other DNA
ttctttaccagactcgagttaagagcttacggtaacctg

SEQ ID NO: 43 - DNA, 42 bp, synthetic construct; identical to SEQ ID NO: 33
  source 1..42: mol_type = other DNA

SEQ ID NO: 44 - DNA, 40 bp, synthetic construct
  source 1..40: mol_type = other DNA
ttctttaccagactcgagttaagagcttacggtaacgaga

SEQ ID NO: 45 - DNA, 41 bp, synthetic construct; identical to SEQ ID NO: 29
  source 1..41: mol_type = other DNA

SEQ ID NO: 46 - DNA, 39 bp, synthetic construct; identical to SEQ ID NO: 42
  source 1..39: mol_type = other DNA

SEQ ID NO: 47 - DNA, 42 bp, synthetic construct; identical to SEQ ID NO: 33
  source 1..42: mol_type = other DNA

SEQ ID NO: 48 - DNA, 39 bp, synthetic construct; identical to SEQ ID NO: 40
  source 1..39: mol_type = other DNA

SEQ ID NO: 49 - protein, 23 aa, synthetic construct
KVDVIDLTIESSSDEEEDPPAKR

SEQ ID NO: 50 - protein, 92 aa, synthetic construct
MSEEKPKEGVKTENDHINLKVAGQDGSVVQFKIKRHTPLSKLMKAYCERQGLSMRQIRFRFDGQPINETDTPAQLEMEDEDTIDVFQQQTVV

SEQ ID NO: 51 - protein, 14 aa, synthetic construct
KKTPPPVPPRTTSK

SEQ ID NO: 52 - protein, 63 aa, synthetic construct
DLNMPAYVKFNYMAEREDELSLIKGTKVIVMEKSSDGWWRGSYNGQVGWFPSNYVTEEGDSPL

SEQ ID NO: 53 - protein, 122 aa, synthetic construct
EVQLLESGGGLVQPGGSLRLSCAASGTFDKINNMGWYRQAPGKQRDLVAQITPGGITDYADSVKGRFTISRDNSKNTLYLQMNSLRPEDTAVYYCNAEILKRAYIDVYVNYWGQGTLVTVSS

SEQ ID NO: 54 - protein, 128 aa, synthetic construct
EVQLMESGGGLVQAGGSLRLSCAASGRTFNNYAMGWFRRAPKGEREFVAAITRSGVRSGVSAIYGDSVKDRFTISRDNAKNTLYLQMNSLKPEDTAVYTCAASAIGSGALRRFEYDYSGQGTQVTVSS